European Patent Application EP 4 417 618 A1, published August 21, 2024. Title: EPHA2 BICYCLIC PEPTIDE LIGAND AND CONJUGATE THEREOF. Applicant: Haisco Pharmaceutical Group Co., Ltd. The sequence listing filed with the application follows.

SEQUENCE LISTING (14 sequences)

SEQ ID NO: 1 - protein, 15 aa, synthetic construct
  SITE 1: note = X stands for Hcys
  SITE 2: note = X stands for Hyp
  SITE 8: note = X stands for Hcys
  SITE 12: note = X stands for D-Asp
  SITE 14: note = X stands for hArg
  SITE 15: note = X stands for Hcys
XXLVNPLXLHPXWXX

SEQ ID NO: 2 - protein, 15 aa, synthetic construct
  SITE 2: note = X stands for Hyp
  SITE 12: note = X stands for D-Asp
  SITE 14: note = X stands for hArg
  SITE 15: note = X stands for Hcys
CXLVNPLCLHPXWXX

SEQ ID NO: 3 - protein, 15 aa, synthetic construct
  SITE 2: note = X stands for Hyp
  SITE 8: note = X stands for Hcys
  SITE 12: note = X stands for D-Asp
  SITE 14: note = X stands for hArg
CXLVNPLXLHPXWXC

SEQ ID NO: 4 - protein, 15 aa, synthetic construct
  SITE 1: note = X stands for Hcys
  SITE 2: note = X stands for Hyp
  SITE 12: note = X stands for D-Asp
  SITE 14: note = X stands for hArg
XXLVNPLCLHPXWXC

SEQ ID NO: 5 - protein, 15 aa, synthetic construct
  SITE 2: note = X stands for Hyp
  SITE 8: note = X stands for Hcys
  SITE 12: note = X stands for D-Asp
  SITE 14: note = X stands for hArg
  SITE 15: note = X stands for Hcys
CXLVNPLXLHPXWXX

SEQ ID NO: 6 - protein, 15 aa, synthetic construct
  SITE 1: note = X stands for Hcys
  SITE 2: note = X stands for Hyp
  SITE 12: note = X stands for D-Asp
  SITE 14: note = X stands for hArg
  SITE 15: note = X stands for Hcys
XXLVNPLCLHPXWXX

SEQ ID NO: 7 - protein, 15 aa, synthetic construct
  SITE 1: note = X stands for Hcys
  SITE 2: note = X stands for Hyp
  SITE 8: note = X stands for Hcys
  SITE 12: note = X stands for D-Asp
  SITE 14: note = X stands for hArg
XXLVNPLXLHPXWXC

SEQ ID NO: 8 - protein, 20 aa, synthetic construct
  SITE 1: note = X stands for beta Ala
  SITE 2: note = X stands for Sar10
  SITE 4: note = X stands for hArg
  SITE 6: note = X stands for Hcys
  SITE 7: note = X stands for Hyp
  SITE 13: note = X stands for Hcys
  SITE 17: note = X stands for D-Asp
  SITE 19: note = X stands for hArg
  SITE 20: note = X stands for Hcys
  SITE 20: note = X stands for Hcys
XXAXDXXLVNPLXLHPXWXX

SEQ ID NO: 9 - protein, 20 aa, synthetic construct
  SITE 1: note = X is beta Ala
  SITE 2: note = X is Sar10
  SITE 4: note = X is hArg
  SITE 7: note = X is Hyp
  SITE 17: note = X is D-Asp
  SITE 19: note = X is hArg
  SITE 20: note = X is Hcys
XXAXDCXLVNPLCLHPXWXX

SEQ ID NO: 10 - protein, 20 aa, synthetic construct
  SITE 1: note = X stands for beta Ala
  SITE 2: note = X stands for Sar10
  SITE 4: note = X stands for hArg
  SITE 7: note = X stands for Hyp
  SITE 13: note = X stands for Hcys
  SITE 17: note = X stands for D-Asp
  SITE 19: note = X stands for hArg
XXAXDCXLVNPLXLHPXWXC

SEQ ID NO: 11 - protein, 20 aa, synthetic construct
  SITE 1: note = X stands for beta Ala
  SITE 2: note = X stands for Sar10
  SITE 4: note = X stands for hArg
  SITE 6: note = X stands for Hcys
  SITE 7: note = X stands for Hyp
  SITE 17: note = X stands for D-Asp
  SITE 19: note = X stands for hArg
XXAXDXXLVNPLCLHPXWXC

SEQ ID NO: 12 - protein, 20 aa, synthetic construct
  SITE 1: note = X stands for beta Ala
  SITE 2: note = X stands for Sar10
  SITE 4: note = X stands for hArg
  SITE 7: note = X stands for Hyp
  SITE 13: note = X stands for Hcys
  SITE 17: note = X stands for D-Asp
  SITE 19: note = X stands for hArg
  SITE 20: note = X stands for Hcys
XXAXDCXLVNPLXLHPXWXX

SEQ ID NO: 13 - protein, 20 aa, synthetic construct
  SITE 1: note = X stands for beta Ala
  SITE 2: note = X stands for Sar10
  SITE 4: note = X stands for hArg
  SITE 6: note = X stands for Hcys
  SITE 7: note = X stands for Hyp
  SITE 17: note = X stands for D-Asp
  SITE 19: note = X stands for hArg
  SITE 20: note = X stands for Hcys
XXAXDXXLVNPLCLHPXWXX

SEQ ID NO: 14 - protein, 20 aa, synthetic construct
  SITE 1: note = X stands for beta Ala
  SITE 2: note = X stands for Sar10
  SITE 4: note = X stands for hArg
  SITE 6: note = X stands for Hcys
  SITE 7: note = X stands for Hyp
  SITE 13: note = X stands for Hcys
  SITE 17: note = X stands for D-Asp
  SITE 19: note = X stands for hArg
XXAXDXXLVNPLXLHPXWXC